European Patent Specification EP 4 114 172 B1, published May 6, 2026. Title: Animal model for hyperkeratosis and sepsis. Applicant: Christian-Albrechts-Universität zu Kiel. The sequence listing filed with the application follows.

SEQUENCE LISTING (4 sequences)

SEQ ID NO: 1 - DNA, 9150 bp, Artificial Sequence
  nucleic acid construct for for overexpressing meprin α
  misc_feature 1..22: /note="forward primer for genotyping"
  misc_feature 1..204: /note="sequence of homology to Rosa26 locus"
  misc_feature 366..387: /note="reverse primer for genotyping"
  promoter 989..1576: /note="CAG promoter"
  misc_recomb 2021..2054: /note="LoxP site"
  misc_feature 2116..2919: /note="neomycin resistance"
  misc_feature 2117..4514: /note="Westphal stop sequence (STOP cassette) "
  misc_recomb 4527..4560: /note="LoxP site"
  CDS 4573..6852: /product="meprin α" /transl_table=1
  CDS 6853..6906: /product="HA tag" /transl_table=1
  CDS 7590..8309: /product="EGFP" /transl_table=1
  misc_feature 8757..9150: /note="sequence of homology to Rosa26 locus"
  misc_feature 9120..9140: /note="reverse primer for genotyping"
aaagtcgctctgagttgttatcagtaagggagctgcagtggagtaggcggggagaaggccgcacccttctccggaggggggaggggagtgttgcaatacctttctgggagttctctgctgcctcctggcttctgaggaccgccctgggcctgggagaatcccttccccctcttccctcgtgatctgcaactccagtctttctagcatctgtagggcgcagtagtccagggtttccttgatgatgtcatacttatcctgtcccttttttttccacagctcgcggttgaggacaaactcttcgcggtctttccagtggttaattaaagttataatcgctgaggtaatatttaaaatcattttcaaatgattcacagttaatttgcgacaatataattttattttcacataaactagacgccttgtcgtcttcttcttcgtattccttctctttttcatttttctcttcataaaaattaacatagttattatcgtatccatatatgtatctatcgtatagagtaaattttttgttgtcataaatatatatgtcttttttaatggggtgtatagtaccgctgcgcatagtttttctgtaatttacaacagtgctattttctggtagttcttcggagtgtgttgctttaattattaaatttatataatcaatgaatttgggatcgtcggttttgtacaatatgttgccggcatagtacgcagcttcttctagttcaattacaccattttttagcagcaccggattaacataactttccaaaatgttgtacgaaccgttaaacaaaaacagttcacctcccttttctatactattgtctgcgagcagttgtttgttgttaaaaataacagccattgtaatgagacgcacaaactaatatcacaaactggaaatgtctatcaatatatagttgctctagttattaatagtaatcaattacggggtcattagttcatagcccatatatggagttccgcgttacataacttacggtaaatggcccgcctggctgaccgcccaacgacccccgcccattgacgtcaataatgacgtatgttcccatagtaacgccaatagggactttccattgacgtcaatgggtggactatttacggtaaactgcccacttggcagtacatcaagtgtatcatatgccaagtacgccccctattgacgtcaatgacggtaaatggcccgcctggcattatgcccagtacatgaccttatgggactttcctacttggcagtacatctacgtattagtcatcgctattaccatgcatggtcgaggtgagccccacgttctgcttcactctccccatctcccccccctccccacccccaattttgtatttatttattttttaattattttgtgcagcgatgggggcggggggggggggggggcgcgcgccaggcggggcggggcggggcgaggggcggggcggggcgaggcggagaggtgcggcggcagccaatcagagcggcgcgctccgaaagtttccttttatggcgaggcggcggcggcggcggccctataaaaagcgaagcgcgcggcgggcgggagtcgctgcgacgctgccttcgccccgtgccccgctccgccgccgcctcgcgccgcccgccccggctctgactgaccgcgttactcccacaggtgagcgggcgggacggcccttctccttcgggctgtaattagcgcttggtttaatgacggcttgtttcttttctgtggctgcgtgaaagccttgaggggctccgggagggccctttgtgcggggggagcggctcggggctgtccgcggggggacggctgccttcgggggggacggggcagggcggggttcggcttctggcgtgtgaccggcggctctagagcctcgctagcatctgtagggcgcagtagtccagggtttccttgatgatgtcatacttatcctgtcccttttttttccacagctcgcggttgaggacaaactcttcgcggtctttccagtggttaattaaataacttcgtatagcatacattatacgaagttatggatccgaacaaacgacccaacacccgtgcgttttattctgtctttttattgccgatcccctcagaagaactcgtcaagaaggcgatagaaggcgatgcgctgcgaatcgggagcggcgataccgtaaagcacgaggaagcggtcagcccattcgccgccaagctcttcagcaatatcacgggtagccaacgctatgtcctgatagcggtccgccacacccagccggccacagtcgatgaatccagaaaagcggccattttccaccatgatattcggcaagcaggcatcgccatgggtcacgacgagatcctcgccgtcgggcatgcgcgccttgagcctggcgaacagttcggctggcgcgagcccctgatgctcttcgtccagatcatcctgatcgacaagaccggcttccatccgagtacgtgctcgctcgatgcgatgtttcgcttggtggtcgaatgggcaggtagccggatcaagcgtatgcagccgccgcattgcatcagccatgatggatactttctcggcaggagcaaggtgagatgacaggagatcctgccccggcacttcgcccaatagcagccagtcccttcccgcttcagtgacaacgtcgagcacagctgcgcaaggaacgcccgtcgtggccagccacgatagccgcgctgcctcgtcctgcagttcattcagggcaccggacaggtcggtcttgacaaaaagaaccgggcgcccctgcgctgacagccggaacacggcggcatcagagcagccgattgtctgttgtgcccagtcatagccgaatagcctctccacccaagcggccggagaacctgcgtgcaatccatcttgttcaatggccgatcccatattggctgcagggtcgctcggtgttcgaggccacacgcgtcaccttaatatgcgaagtggacctgggaccgcgccgccccgactgcatctgcgtgttcgaattcgccaatgacaagacgctgggcggggtttgctcgacattgggtggaaacattccaggcctgggtggagaggctttttgcttcctcttgcaaaaccacactgctcgacattgggtggaaacattccaggcctgggtggagaggctttttgcttcctcttgcaaaaccacactgctcgactagtgattaaagtcgactcggggacaccaaatatggcgatctcggccttttcgtttcttggagctgggacatgtttgccatcgatccatctaccaccagaacggccgttagatctgctgccaccgttgtttccaccgaagaaaccaccgttgccgtaaccaccacgacggttgttgctaaagaagctgccaccgccacggccaccgttgtagccgccgttgttgttattgtagttgctcatgttatttctggcacttcttggttttcctcttaagtgaggaggaacataaccattctcgttgttgtcgttgatgcttaaattttgcacttgttcgctcagttcagccataatatgaaatgcttttcttgttgttcttacggaataccacttgccacctatcaccacaactaactttttcccgttcctccatctcttttatattttttttctcgagggatctttgtgaaggaaccttacttctgtggtgtgacataattggacaaactacctacagagatttaaagctctaaggtaaatataaaatttttaagtgtataatgtgttaaactactgattctaattgtttgtgtattttagattccaacctatggaactgatgaatgggagcagtggtggaatgcctttaatgaggaaaacctgttttgctcagaagaaatgccatctagtgatgatgaggctactgctgactctcaacattctactcctccaaaaaagaagagaaaggtagaagaccccaaggactttccttcagaattgctaagttttttgagtcatgctgtgtttagtaatagaactcttgcttgctttgctatttacaccacaaaggaaaaagctgcactgctatacaagaaaattatggaaaaatattctgtaacctttataagtaggcataacagttataatcataacatactgttttttcttactccacacaggcatagagtgtctgctattaataactatgctcaaaaattgtgtacctttagctttttaatttgtaaaggggttaataaggaatatttgatgtatagtgccttgactagagatcataatcagccataccacatttgtagaggttttacttgctttaaaaaacctcccacacctccccctgaacctgaaacataaaatgaatgcaattgttgttgttaacttgtttattgcagcttataatggttacaaataaagcaatagcatcacaaatttcacaaataaagcatttttttcactgcattctagttgtggtttgtccaaactcatcaatgtatcttatcatgtctggatctgacatggtaagtaagcttataacttcgtatagcatacattatacgaagttatcggcgcgccaccatggcaaggaggcttggcagatccagttcatttgcaataatgctttggatacaacctgcgtgtcttctctcactgattttttctgcccacatagcagctgtatcgattaagcatcttttgaatggatctgatcacgatacagatgttggtgaacagaaggatattttcgaaatcaatttagctgcaggcctgaacctctttcaaggggacatccttctgcccagaaccagaaatgccatgcgagatccctcaagcagatggaagctccccattccatacattctggctgacaatctggagctgaatgccaaaggagccatcctccatgcctttgagatgttccgcctcaagtcttgtgtggatttcaagccctacgaaggggagagttcgtatatcatcttccagaaactttctgggtgctggtctatgattggtgatcaacaggtgggacagaacatttccattggtgagggatgtgactttaaggccaccattgaacatgaaatcctgcatgctctgggattcttccatgagcagtcaaggactgaccgggatgattatgtgaacatttggtgggatcaaatcattacagactatgaacataatttcaacacatatgacgacaacaccatcacagacctcaacacaccctatgattatgagtccctgatgcactacgggccattttcgtttaacaagaacgaaagcatccctaccattactaccaagatccctgagtttaacaccatcattggacaactcccggacttcagtgccattgatctaataagactgaatcgaatgtacaactgcaccgcaacacatactctgttggaccactgtgactttgagaagaccaacgtctgtgggatgatccagggaaccagagatgatgctgattgggctcatggggacagcagtcagcctgaacaagtggatcacaccttggtgggacagtgtaaaggtgccggctacttcatgttcttcaataccagcttgggggcaagaggagaggcagcccttctggagtctcgaatcctttatcccaagaggaagcagcagtgtttgcagtttttttataagatgactggaagccctgcagacagatttgaagtctgggtgagaagggacgacaacgcgggcaaggtgcgacagctggccaagatccagacctttcaaggagactctgatcacaactggaaaattgctcatgtgacactcaatgaagaaaagaaatttcgctatgttttcctgggtaccaaaggggaccctggtaactcaagtggtggtatttaccttgatgacatcactctgacagaaaccccctgccctgcaggggtttggaccatccggaatatctcccagatccttgagaacacagtgaaaggggacaagctcgtgagccctcggttctacaattctgagggttacggtgtgggggtgaccttgtaccccaatggtagaatcaccagtaactctggcttcctgggactcacttttcacttgtacagtggggataacgatgcgattctggagtggccagtggaaaacagacaggccataatgaccatcctggaccaggaagctgataccaggaacaggatgtccctgaccttgatgttcactacctccaagaaccaaacatcttcagctataaatggctctgtcatctgggacaggccatccaaggtgggagtctatgataaggactgtgattgtttcagaagccttgactggggctggggtcaggccatctcccaccagctgctgaagagaagaaattttcttaaaggcgacagcctcatcattttcgtggactttaaagacctcacccacctgaaccggactgaagttccagcttcagccagaagcacgatgcccagaggcctccttctgcaaggccaggagtctcctgccttgggagaaagctccagaaaagccatgctggaggaatccctgccaagcagcctgggccagagacatcccagcagacagaagcgctcggtggagaacactggccccatggaggaccacaactggccacagtacttcagagacccctgtgacccaaacccttgccagaatgaaggcacctgtgtgaacgtaaagggaatggccagctgcaggtgcgtctctgggcacgcctttttctacgcaggggagcgctgtcaggccatgcacgtgcacggcagcttgctgggcctgctcattggctgcatcgctggcttgatcttcttgaccttcgtcacattctctaccaccaacggaaagctgcggcagtacccatacgacgtcccagactacgcttacccatacgacgtcccagactacgcttgaggcgcgccgcggccgcgatcaattcggtaccgaagttcctattccgaagttcctattctctagaaagtataggaacttcctcgagggtaccccaattccgccccccccccccccctaacgttactggccgaagccgcttggaataaggccggtgtgcgtttgtctatatgttattttccaccatattgccgtcttttggcaatgtgagggcccggaaacctggccctgtcttcttgacgagcattcctaggggtctttcccctctcgccaaaggaatgcaaggtctgttgaatgtcgtgaaggaagcagttcctctggaagcttcttgaagacaaacaacgtctgtagcgaccctttgcaggcagcggaaccccccacctggcgacaggtgcctctgcggccaaaagccacgtgtataagatacacctgcaaaggcggcacaaccccagtgccacgttgtgagttggatagttgtggaaagagtcaaatggctctcctcaagcgtattcaacaaggggctgaaggatgcccagaaggtaccccattgtatgggatctgatctggggcctcggtgcacatgctttacatgtgtttagtcgaggttaaaaaacgtctaggccccccgaaccacggggacgtggttttcctttgaaaaacacgatgataatatggccacaaccatggtgagcaagggcgaggagctgttcaccggggtggtgcccatcctggtcgagctggacggcgacgtaaacggccacaagttcagcgtgtccggcgagggcgagggcgatgccacctacggcaagctgaccctgaagttcatctgcaccaccggcaagctgcccgtgccctggcccaccctcgtgaccaccctgacctacggcgtgcagtgcttcagccgctaccccgaccacatgaagcagcacgacttcttcaagtccgccatgcccgaaggctacgtccaggagcgcaccatcttcttcaaggacgacggcaactacaagacccgcgccgaggtgaagttcgagggcgacaccctggtgaaccgcatcgagctgaagggcatcgacttcaaggaggacggcaacatcctggggcacaagctggagtacaactacaacagccacaacgtctatatcatggccgacaagcagaagaacggcatcaaggtgaacttcaagatccgccacaacatcgaggacggcagcgtgcagctcgccgaccactaccagcagaacacccccatcggcgacggccccgtgctgctgcccgacaaccactacctgagcacccagtccgccctgagcaaagaccccaacgagaagcgcgatcacatggtcctgctggagttcgtgaccgccgccgggatcactctcggcatggacgagctgtacaagtaatccgggatccggagagctcccaacgaagttcctattccgaagttcctattctctagaaagtataggaacttcctcgaggttggatgcagcccgggggatccactagttctagagcggccgatcagcctcgactgtgccttctagttgccagccatctgttgtttgcccctcccccgtgccttccttgaccctggaaggtgccactcccactgtcctttcctaataaaatgaggaaattgcatcgcattgtctgagtaggtgtcattctattctggggggtggggtggggcaggacagcaagggggaggattgggaagacaatagcaggcatgctggggatgcggtgggctctatggcttctgaggcggaaagaaccagctggggctcgagatccactagttctagcctcgaggctagagcggccgccgcggatatcgaattcgctagaagatgggcgggagtcttctgggcaggcttaaaggctaacctggtgtgtgggcgttgtcctgcaggggaattgaacaggtgtaaaattggagggacaagacttcccacagattttcggttttgtcgggaagttttttaataggggcaaataaggaaaatgggaggataggtagtcatctggggttttatgcagcaaaactacaggttattattgcttgtgatccgcctcggagtattttccatcgaggtagattaaagacatgctcacccgagttttatactctcctgcttgagatccttactacagtatgaaattacagtgtcgcgagttagactatgtaagcagaattttaatcatttttaaagagcccagtacttcatatccatttctccc

SEQ ID NO: 2 - protein, 760 aa, Artificial Sequence
  [CDS]:4573..6852 from SEQ ID NO 1
MARRLGRSSSFAIMLWIQPACLLSLIFSAHIAAVSIKHLLNGSDHDTDVGEQKDIFEINLAAGLNLFQGDILLPRTRNAMRDPSSRWKLPIPYILADNLELNAKGAILHAFEMFRLKSCVDFKPYEGESSYIIFQKLSGCWSMIGDQQVGQNISIGEGCDFKATIEHEILHALGFFHEQSRTDRDDYVNIWWDQIITDYEHNFNTYDDNTITDLNTPYDYESLMHYGPFSFNKNESIPTITTKIPEFNTIIGQLPDFSAIDLIRLNRMYNCTATHTLLDHCDFEKTNVCGMIQGTRDDADWAHGDSSQPEQVDHTLVGQCKGAGYFMFFNTSLGARGEAALLESRILYPKRKQQCLQFFYKMTGSPADRFEVWVRRDDNAGKVRQLAKIQTFQGDSDHNWKIAHVTLNEEKKFRYVFLGTKGDPGNSSGGIYLDDITLTETPCPAGVWTIRNISQILENTVKGDKLVSPRFYNSEGYGVGVTLYPNGRITSNSGFLGLTFHLYSGDNDAILEWPVENRQAIMTILDQEADTRNRMSLTLMFTTSKNQTSSAINGSVIWDRPSKVGVYDKDCDCFRSLDWGWGQAISHQLLKRRNFLKGDSLIIFVDFKDLTHLNRTEVPASARSTMPRGLLLQGQESPALGESSRKAMLEESLPSSLGQRHPSRQKRSVENTGPMEDHNWPQYFRDPCDPNPCQNEGTCVNVKGMASCRCVSGHAFFYAGERCQAMHVHGSLLGLLIGCIAGLIFLTFVTFSTTNGKLRQ

SEQ ID NO: 3 - protein, 18 aa, Artificial Sequence
  [CDS]:6853..6906 from SEQ ID NO 1
YPYDVPDYAYPYDVPDYA

SEQ ID NO: 4 - protein, 239 aa, Artificial Sequence
  [CDS]:7590..8309 from SEQ ID NO 1
MVSKGEELFTGVVPILVELDGDVNGHKFSVSGEGEGDATYGKLTLKFICTTGKLPVPWPTLVTTLTYGVQCFSRYPDHMKQHDFFKSAMPEGYVQERTIFFKDDGNYKTRAEVKFEGDTLVNRIELKGIDFKEDGNILGHKLEYNYNSHNVYIMADKQKNGIKVNFKIRHNIEDGSVQLADHYQQNTPIGDGPVLLPDNHYLSTQSALSKDPNEKRDHMVLLEFVTAAGITLGMDELYK